European Patent Specification EP 3 250 216 B1, published November 8, 2023. Title: composition. Applicant: DuPont Nutrition Biosciences ApS. The sequence listing filed with the application follows.

SEQUENCE LISTING (4 sequences)

SEQ ID NO: 1 - DNA, 20 bp, artificial sequence
  primer
ggactgcagcgtagacgctt

SEQ ID NO: 2 - DNA, 21 bp, artificial sequence
  primer
catcctgtatatgaggcccat

SEQ ID NO: 3 - DNA, 24 bp, Artificial sequence
  Beta-actin Forward primer
gatcaagatcattgctcctcctga

SEQ ID NO: 4 - DNA, 20 bp, artificial sequence
  Beta-actin Reverse primer
cagctcagtaacagtccgcc